European Patent Application EP 4 397 320 A1, published July 10, 2024. Title: RADIOACTIVE COMPLEX OF DEGLYCOSYLATED ANTIBODY AND RADIOACTIVE PHARMACEUTICAL PRODUCT. Applicant: NIHON MEDI-PHYSICS CO., LTD. Application EP 22864604.8, filed August 31, 2022. The sequence listing filed with the application follows.

SEQUENCE LISTING (19 sequences)

SEQ ID NO: 1 - protein, 13 aa, synthetic construct
  REGION 1..13: note = antibody modifying peptide
  SITE 6: note = misc_feature - lysine, cystein, aspartic acid, glutamic acid, 2-aminosuberic acid, or diaminopropionic acid
DCAYHXGELVWCT

SEQ ID NO: 2 - protein, 17 aa, synthetic construct
  REGION 1..17: note = antibody modifying peptide
  SITE 8: note = misc_feature - lysine, cystein, aspartic acid, glutamic acid, 2-aminosuberic acid, or diaminopropionic acid
GPDCAYHXGELVWCTFH

SEQ ID NO: 3 - protein, 13 aa, synthetic construct
  REGION 1..13: note = antibody modifying peptide
  SITE 6: note = misc_feature - lysine, cystein, aspartic acid, glutamic acid, 2-aminosuberic acid, or diaminopropionic acid
RCAYHXGELVWCS

SEQ ID NO: 4 - protein, 17 aa, synthetic construct
  REGION 1..17: note = antibody modifying peptide
  SITE 8: note = misc_feature - lysine, cystein, aspartic acid, glutamic acid, 2-aminosuberic acid, or diaminopropionic acid
GPRCAYHXGELVWCSFH

SEQ ID NO: 5 - protein, 17 aa, synthetic construct
  REGION 1..17: note = antibody modifying peptide
  SITE 8: note = misc_feature - lysine, cystein, aspartic acid, glutamic acid, 2-aminosuberic acid, or diaminopropionic acid
SPDCAYHXGELVWCTFH

SEQ ID NO: 6 - protein, 17 aa, synthetic construct
  REGION 1..17: note = antibody modifying peptide
  SITE 8: note = misc_feature -lysine, cystein, aspartic acid, glutamic acid, 2-aminosuberic acid, or diaminopropionic acid
GDDCAYHXGELVWCTFH

SEQ ID NO: 7 - protein, 17 aa, synthetic construct
  REGION 1..17: note = antibody modifying peptide
  SITE 8: note = misc_feature - lysine, cystein, aspartic acid, glutamic acid, 2-aminosuberic acid, or diaminopropionic acid
GPSCAYHXGELVWCTFH

SEQ ID NO: 8 - protein, 17 aa, synthetic construct
  REGION 1..17: note = antibody modifying peptide
  SITE 8: note = misc_feature - lysine, cystein, aspartic acid, glutamic acid, 2-aminosuberic acid, or diaminopropionic acid
GPDCAYHXGELVWCSFH

SEQ ID NO: 9 - protein, 17 aa, synthetic construct
  REGION 1..17: note = antibody modifying peptide
  SITE 8: note = misc_feature - lysine, cystein, aspartic acid, glutamic acid, 2-aminosuberic acid, or diaminopropionic acid
GPDCAYHXGELVWCTHH

SEQ ID NO: 10 - protein, 17 aa, synthetic construct
  REGION 1..17: note = antibody modifying peptide
  SITE 8: note = misc_feature - lysine, cystein, aspartic acid, glutamic acid, 2-aminosuberic acid, or diaminopropionic acid
GPDCAYHXGELVWCTFY

SEQ ID NO: 11 - protein, 17 aa, synthetic construct
  REGION 1..17: note = antibody modifying peptide
  SITE 8: note = misc_feature -lysine, cystein, aspartic acid, glutamic acid, 2-aminosuberic acid, or diaminopropionic acid
SPDCAYHXGELVWCTFY

SEQ ID NO: 12 - protein, 17 aa, synthetic construct
  REGION 1..17: note = antibody modifying peptide
  SITE 8: note = misc_feature - lysine, cystein, aspartic acid, glutamic acid, 2-aminosuberic acid, or diaminopropionic acid
SDDCAYHXGELVWCTFY

SEQ ID NO: 13 - protein, 17 aa, synthetic construct
  REGION 1..17: note = antibody modifying peptide
  SITE 8: note = misc_feature - lysine, cystein, aspartic acid, glutamic acid, 2-aminosuberic acid, or diaminopropionic acid
RGNCAYHXGQLVWCTYH

SEQ ID NO: 14 - protein, 17 aa, synthetic construct
  REGION 1..17: note = antibody modifying peptide
  SITE 2: note = misc_feature - homocysteine
  SITE 8: note = misc_feature - lysine, cystein, aspartic acid, glutamic acid, 2-aminosuberic acid, or diaminopropionic acid
  SITE 16: note = misc_feature - homocysteine
GXDCAYHXGELVWCTXH

SEQ ID NO: 15 - protein, 13 aa, synthetic construct
  REGION 1..13: note = antibody modifying peptide
  SITE 6: note = misc_feature - lysine, cystein, aspartic acid, glutamic acid, 2-aminosuberic acid, or diaminopropionic acid
DCTYHXGNLVWCT

SEQ ID NO: 16 - protein, 13 aa, synthetic construct
  REGION 1..13: note = antibody modifying peptide
  SITE 6: note = misc_feature - lysine, cystein, aspartic acid, glutamic acid, 2-aminosuberic acid, or diaminopropionic acid
DCAYHXGNLVWCT

SEQ ID NO: 17 - protein, 13 aa, synthetic construct
  REGION 1..13: note = antibody modifying peptide
  SITE 6: note = misc_feature - lysine, cystein, aspartic acid, glutamic acid, 2-aminosuberic acid, or diaminopropionic acid
DCTYHXGELVWCT

SEQ ID NO: 18 - protein, 13 aa, synthetic construct
  REGION 1..13: note = antibody modifying peptide
  SITE 6: note = misc_feature - lysine, cystein, aspartic acid, glutamic acid, 2-aminosuberic acid, or diaminopropionic acid
DCAWHXGELVWCT

SEQ ID NO: 19 - protein, 17 aa, synthetic construct
  DISULFID 4..14: note = Cys-Cys
GPDCAYHKGELVWCTFH